European Patent Application EP 4 282 958 A1, published November 29, 2023. Title: Novel citrate synthase variant and a method for producing L-valine acid using the same. Applicant: CJ CheilJedang Corporation. The sequence listing filed with the application follows.

SEQUENCE LISTING (38 sequences)

SEQ ID NO: 1 - protein, 437 aa, Unknown
  ATCC 14067 GltA AA
MFERDIVATDNNKAVLHYPGGEFEMDIIEASEGNNGVVLGKMLSETGLITFDPGYVSTGSTESKITYIDGDAGILRYRGYDIADLAENATFNEVSYLLINGELPTPDELHKFNDEIRHHTLLDEDFKSQFNVFPRDAHPMATLASSVNILSTYYQDQLNPLDEAQLDKATVRLMAKVPMLAAYAHRARKGAPYMYPDNSLNARENFLRMMFGYPTEPYEIDPIMVKALDKLLILHADHEQNCSTSTVRMIGSAQANMFVSIAGGINALSGPLHGGANQAVLEMLEDIKNNHGGDATAFMNKVKNKEDGVRLMGFGHRVYKNYDPRAAIVKETAHEILEHLGGDDLLDLAIKLEEIALADDYFISRKLYPNVDFYTGLIYRAMGFPTDFFTVLFAIGRLPGWIAHYREQLGAAGNKINRPRQVYTGNESRKLVPREER

SEQ ID NO: 2 - DNA, 1314 bp, Unknown
  ATCC 14067 GltA NT
atgtttgaaagggatatcgtggctactgataacaacaaggctgtcctgcactaccccggtggcgagttcgaaatggacatcatcgaggcttctgagggtaacaacggtgttgtcctgggcaagatgctgtctgagactggactgatcacttttgacccaggttatgtgagcactggctccaccgagtcgaagatcacctacatcgatggcgatgcgggaatcctgcgttaccgcggctatgacatcgctgatctggctgagaatgccaccttcaacgaggtttcttacctacttatcaacggtgagctaccaaccccagatgagcttcacaagtttaacgacgagattcgccaccacacccttctggacgaggacttcaagtcccagttcaacgtgttcccacgcgacgctcacccaatggcaaccttggcttcctcggttaacattttgtctacctactaccaggatcagctgaacccactcgatgaggcacagcttgataaggcaaccgttcgcctcatggcaaaggttccaatgctggctgcgtacgcacaccgcgcacgcaagggtgctccttacatgtacccagacaactccctcaacgcgcgtgagaacttcctgcgcatgatgttcggttacccaactgagccatacgagatcgacccaatcatggtcaaggctctggacaagctgctcatcctgcacgctgaccacgagcagaactgctccacctccaccgttcgtatgatcggttccgcacaggccaacatgtttgtctccatcgctggtggcatcaacgctctgtccggcccactgcacggtggcgcaaaccaggctgttctggagatgctcgaagacatcaagaacaaccacggtggcgacgcaaccgcgttcatgaacaaggtcaagaacaaggaagacggcgtccgcctcatgggcttcggacaccgcgtttacaagaattacgatccacgtgcagcaatcgtcaaggagaccgcacacgagatcctcgagcacctcggtggcgacgatcttctggatctggcaatcaagctggaagaaattgcactggctgatgattacttcatctcccgcaagctctacccgaacgtagacttctacaccggcctgatctaccgcgcaatgggcttcccaactgacttcttcaccgtattgttcgcaatcggtcgtctgccaggatggatcgctcactaccgcgagcagctcggtgcagcaggcaacaagatcaaccgcccacgccaggtctacaccggcaacgaatcccgcaagttggttcctcgcgaggagcgctaa

SEQ ID NO: 3 - protein, 52 aa, Unknown
  ATCC 14067 GltA 362~413
FISRKLYPNVDFYTGLIYRAMGFPTDFFTVLFAIGRLPGWIAHYREQLGAAD

SEQ ID NO: 4 - protein, 437 aa, Unknown [sequence omitted]

SEQ ID NO: 5 - DNA, 1314 bp, Unknown
  ATCC13032 GltA NT
atgtttgaaagggatatcgtggctactgataacaacaaggctgtcctgcactaccccggtggcgagttcgaaatggacatcatcgaggcttctgagggtaacaacggtgttgtcctgggcaagatgctgtctgagactggactgatcacttttgacccaggttatgtgagcactggctccaccgagtcgaagatcacctacatcgatggcgatgcgggaatcctgcgttaccgcggctatgacatcgctgatctggctgagaatgccaccttcaacgaggtttcttacctacttatcaacggtgagctaccaaccccagatgagcttcacaagtttaacgacgagattcgccaccacacccttctggacgaggacttcaagtcccagttcaacgtgttcccacgcgacgctcacccaatggcaaccttggcttcctcggttaacattttgtctacctactaccaggaccagctgaacccactcgatgaggcacagcttgataaggcaaccgttcgcctcatggcaaaggttccaatgctggctgcgtacgcacaccgcgcacgcaagggtgctccttacatgtacccagacaactccctcaatgcgcgtgagaacttcctgcgcatgatgttcggttacccaaccgagccatacgagatcgacccaatcatggtcaaggctctggacaagctgctcatcctgcacgctgaccacgagcagaactgctccacctccaccgttcgtatgatcggttccgcacaggccaacatgtttgtctccatcgctggtggcatcaacgctctgtccggcccactgcacggtggcgcaaaccaggctgttctggagatgctcgaagacatcaagagcaaccacggtggcgacgcaaccgagttcatgaacaaggtcaagaacaaggaagacggcgtccgcctcatgggcttcggacaccgcgtttacaagaactacgatccacgtgcagcaatcgtcaaggagaccgcacacgagatcctcgagcacctcggtggcgacgatcttctggatctggcaatcaagctggaagaaattgcactggctgatgattacttcatctcccgcaagctctacccgaacgtagacttctacaccggcctgatctaccgcgcaatgggcttcccaactgacttcttcaccgtattgttcgcaatcggtcgtctgccaggatggatcgctcactaccgcgagcagctcggtgcagcaggcaacaagatcaaccgcccacgccaggtctacaccggcaacgaatcccgcaagttggttcctcgcgaggagcgctaa

SEQ ID NO: 6 - protein, 437 aa, Unknown
  ATCC13869 GltA AA
MFERDIVATDNNKAVLHYPGGEFEMDIIEASEGNNGVVLGKMLSETGLITFDPGYVSTGSTESKITYIDGDAGILRYRGYDIADLAENATFNEVSYLLINGELPTPDELHKFNDEIRHHTLLDEDFKSQFNVFPRDAHPMATLASSVNILSTYYQDQLNPLDEAQLDKATVRLMAKVPMLAAYAHRARKGAPYMYPDNSLNARENFLRMMFGYPTEPYEIDPIMVKALDKLLILHADHEQNCSTSTVRMIGSAQANMFVSIAGGINALSGPLHGGANQAVLEMLEDIKNNHGGDATAFMNKVKNKEDGVRLMGFGHRVYKNYDPRAAIVKETAHEILEHLGGDDLLDLAIKLEEIALADDCFISRKLYPNVDFYTGLIYRAMGFPTDFFTVLFAIGRLPGWIAHYREQLGAAGNKINRPRQVYTGKESRKLVPREER

SEQ ID NO: 7 - DNA, 1314 bp, Unknown
  ATCC13869 GltA NT
atgtttgaaagggatatcgtggctactgataacaacaaggctgtcctgcactaccccggtggcgagttcgaaatggacatcatcgaggcttctgagggtaacaacggtgttgtcctgggcaagatgctgtctgagactggactgatcacttttgacccaggttatgtgagcactggctccaccgagtcgaagatcacctacatcgatggcgatgcgggaatcctgcgttaccgcggctatgacatcgctgatctggctgagaatgccaccttcaacgaggtttcttacctacttatcaacggtgagctaccaaccccagatgagcttcacaagtttaacgacgagattcgccaccacacccttctggacgaggacttcaagtcccagttcaacgtgttcccacgcgacgctcacccaatggcaaccttggcttcctcggttaacattttgtctacctactaccaggatcagctgaacccactcgatgaggcacagcttgataaggcaaccgttcgcctcatggcaaaggttccaatgctggctgcgtacgcacaccgcgcacgcaagggtgctccttacatgtacccagacaactccctcaacgcgcgtgagaacttcctgcgcatgatgttcggttacccaaccgagccatacgagatcgacccaatcatggtcaaggctctggacaagctgctcatcctgcacgctgaccacgagcagaactgctccacctccaccgttcgtatgatcggttccgcacaggccaacatgtttgtctccatcgctggtggcatcaacgctctgtccggcccactgcacggtggcgcaaaccaggctgttctggagatgctcgaagacatcaagaacaaccacggtggcgacgcaaccgcgttcatgaacaaggtcaagaacaaggaagacggcgtccgcctcatgggcttcggacaccgcgtttacaagaactacgatccacgtgcagcaatcgtcaaggagaccgcacacgagatcctcgagcacctcggtggcgacgatcttctggatctggcaatcaagctggaagaaattgcactggctgatgattgcttcatctcccgcaagctctacccgaacgtagacttctacaccggcctgatctaccgcgcaatgggcttcccaactgacttcttcaccgtattgttcgcaatcggtcgtctgccaggatggatcgctcactaccgcgagcagctcggtgcagcaggcaacaagatcaaccgcccacgccaggtctacaccggcaaggaatcccgcaagttggttcctcgcgaggagcgctaa

SEQ ID NO: 8 - protein, 437 aa, Artificial Sequence
  ATCC 14067 GltA G413D AA
MFERDIVATDNNKAVLHYPGGEFEMDIIEASEGNNGVVLGKMLSETGLITFDPGYVSTGSTESKITYIDGDAGILRYRGYDIADLAENATFNEVSYLLINGELPTPDELHKFNDEIRHHTLLDEDFKSQFNVFPRDAHPMATLASSVNILSTYYQDQLNPLDEAQLDKATVRLMAKVPMLAAYAHRARKGAPYMYPDNSLNARENFLRMMFGYPTEPYEIDPIMVKALDKLLILHADHEQNCSTSTVRMIGSAQANMFVSIAGGINALSGPLHGGANQAVLEMLEDIKNNHGGDATAFMNKVKNKEDGVRLMGFGHRVYKNYDPRAAIVKETAHEILEHLGGDDLLDLAIKLEEIALADDYFISRKLYPNVDFYTGLIYRAMGFPTDFFTVLFAIGRLPGWIAHYREQLGAADNKINRPRQVYTGNESRKLVPREER

SEQ ID NO: 9 - DNA, 1314 bp, Artificial Sequence
  ATCC 14067 GltA G413D  NT
atgtttgaaagggatatcgtggctactgataacaacaaggctgtcctgcactaccccggtggcgagttcgaaatggacatcatcgaggcttctgagggtaacaacggtgttgtcctgggcaagatgctgtctgagactggactgatcacttttgacccaggttatgtgagcactggctccaccgagtcgaagatcacctacatcgatggcgatgcgggaatcctgcgttaccgcggctatgacatcgctgatctggctgagaatgccaccttcaacgaggtttcttacctacttatcaacggtgagctaccaaccccagatgagcttcacaagtttaacgacgagattcgccaccacacccttctggacgaggacttcaagtcccagttcaacgtgttcccacgcgacgctcacccaatggcaaccttggcttcctcggttaacattttgtctacctactaccaggatcagctgaacccactcgatgaggcacagcttgataaggcaaccgttcgcctcatggcaaaggttccaatgctggctgcgtacgcacaccgcgcacgcaagggtgctccttacatgtacccagacaactccctcaacgcgcgtgagaacttcctgcgcatgatgttcggttacccaactgagccatacgagatcgacccaatcatggtcaaggctctggacaagctgctcatcctgcacgctgaccacgagcagaactgctccacctccaccgttcgtatgatcggttccgcacaggccaacatgtttgtctccatcgctggtggcatcaacgctctgtccggcccactgcacggtggcgcaaaccaggctgttctggagatgctcgaagacatcaagaacaaccacggtggcgacgcaaccgcgttcatgaacaaggtcaagaacaaggaagacggcgtccgcctcatgggcttcggacaccgcgtttacaagaattacgatccacgtgcagcaatcgtcaaggagaccgcacacgagatcctcgagcacctcggtggcgacgatcttctggatctggcaatcaagctggaagaaattgcactggctgatgattacttcatctcccgcaagctctacccgaacgtagacttctacaccggcctgatctaccgcgcaatgggcttcccaactgacttcttcaccgtattgttcgcaatcggtcgtctgccaggatggatcgctcactaccgcgagcagctcggtgcagcagacaacaagatcaaccgcccacgccaggtctacaccggcaacgaatcccgcaagttggttcctcgcgaggagcgctaa

SEQ ID NO: 10 - protein, 437 aa, Artificial Sequence
  ATCC13032 GltA G413D AA
MFERDIVATDNNKAVLHYPGGEFEMDIIEASEGNNGVVLGKMLSETGLITFDPGYVSTGSTESKITYIDGDAGILRYRGYDIADLAENATFNEVSYLLINGELPTPDELHKFNDEIRHHTLLDEDFKSQFNVFPRDAHPMATLASSVNILSTYYQDQLNPLDEAQLDKATVRLMAKVPMLAAYAHRARKGAPYMYPDNSLNARENFLRMMFGYPTEPYEIDPIMVKALDKLLILHADHEQNCSTSTVRMIGSAQANMFVSIAGGINALSGPLHGGANQAVLEMLEDIKSNHGGDATEFMNKVKNKEDGVRLMGFGHRVYKNYDPRAAIVKETAHEILEHLGGDDLLDLAIKLEEIALADDYFISRKLYPNVDFYTGLIYRAMGFPTDFFTVLFAIGRLPGWIAHYREQLGAADNKINRPRQVYTGNESRKLVPREER

SEQ ID NO: 11 - DNA, 1314 bp, Artificial Sequence
  ATCC13032 GltA G413D NT
atgtttgaaagggatatcgtggctactgataacaacaaggctgtcctgcactaccccggtggcgagttcgaaatggacatcatcgaggcttctgagggtaacaacggtgttgtcctgggcaagatgctgtctgagactggactgatcacttttgacccaggttatgtgagcactggctccaccgagtcgaagatcacctacatcgatggcgatgcgggaatcctgcgttaccgcggctatgacatcgctgatctggctgagaatgccaccttcaacgaggtttcttacctacttatcaacggtgagctaccaaccccagatgagcttcacaagtttaacgacgagattcgccaccacacccttctggacgaggacttcaagtcccagttcaacgtgttcccacgcgacgctcacccaatggcaaccttggcttcctcggttaacattttgtctacctactaccaggaccagctgaacccactcgatgaggcacagcttgataaggcaaccgttcgcctcatggcaaaggttccaatgctggctgcgtacgcacaccgcgcacgcaagggtgctccttacatgtacccagacaactccctcaatgcgcgtgagaacttcctgcgcatgatgttcggttacccaaccgagccatacgagatcgacccaatcatggtcaaggctctggacaagctgctcatcctgcacgctgaccacgagcagaactgctccacctccaccgttcgtatgatcggttccgcacaggccaacatgtttgtctccatcgctggtggcatcaacgctctgtccggcccactgcacggtggcgcaaaccaggctgttctggagatgctcgaagacatcaagagcaaccacggtggcgacgcaaccgagttcatgaacaaggtcaagaacaaggaagacggcgtccgcctcatgggcttcggacaccgcgtttacaagaactacgatccacgtgcagcaatcgtcaaggagaccgcacacgagatcctcgagcacctcggtggcgacgatcttctggatctggcaatcaagctggaagaaattgcactggctgatgattacttcatctcccgcaagctctacccgaacgtagacttctacaccggcctgatctaccgcgcaatgggcttcccaactgacttcttcaccgtattgttcgcaatcggtcgtctgccaggatggatcgctcactaccgcgagcagctcggtgcagcagacaacaagatcaaccgcccacgccaggtctacaccggcaacgaatcccgcaagttggttcctcgcgaggagcgctaa

SEQ ID NO: 12 - protein, 437 aa, Artificial Sequence
  ATCC13869 GltA G413D AA
MFERDIVATDNNKAVLHYPGGEFEMDIIEASEGNNGVVLGKMLSETGLITFDPGYVSTGSTESKITYIDGDAGILRYRGYDIADLAENATFNEVSYLLINGELPTPDELHKFNDEIRHHTLLDEDFKSQFNVFPRDAHPMATLASSVNILSTYYQDQLNPLDEAQLDKATVRLMAKVPMLAAYAHRARKGAPYMYPDNSLNARENFLRMMFGYPTEPYEIDPIMVKALDKLLILHADHEQNCSTSTVRMIGSAQANMFVSIAGGINALSGPLHGGANQAVLEMLEDIKNNHGGDATAFMNKVKNKEDGVRLMGFGHRVYKNYDPRAAIVKETAHEILEHLGGDDLLDLAIKLEEIALADDCFISRKLYPNVDFYTGLIYRAMGFPTDFFTVLFAIGRLPGWIAHYREQLGAADNKINRPRQVYTGKESRKLVPREER

SEQ ID NO: 13 - DNA, 1314 bp, Artificial Sequence
  ATCC13869 GltA G413D NT
atgtttgaaagggatatcgtggctactgataacaacaaggctgtcctgcactaccccggtggcgagttcgaaatggacatcatcgaggcttctgagggtaacaacggtgttgtcctgggcaagatgctgtctgagactggactgatcacttttgacccaggttatgtgagcactggctccaccgagtcgaagatcacctacatcgatggcgatgcgggaatcctgcgttaccgcggctatgacatcgctgatctggctgagaatgccaccttcaacgaggtttcttacctacttatcaacggtgagctaccaaccccagatgagcttcacaagtttaacgacgagattcgccaccacacccttctggacgaggacttcaagtcccagttcaacgtgttcccacgcgacgctcacccaatggcaaccttggcttcctcggttaacattttgtctacctactaccaggatcagctgaacccactcgatgaggcacagcttgataaggcaaccgttcgcctcatggcaaaggttccaatgctggctgcgtacgcacaccgcgcacgcaagggtgctccttacatgtacccagacaactccctcaacgcgcgtgagaacttcctgcgcatgatgttcggttacccaaccgagccatacgagatcgacccaatcatggtcaaggctctggacaagctgctcatcctgcacgctgaccacgagcagaactgctccacctccaccgttcgtatgatcggttccgcacaggccaacatgtttgtctccatcgctggtggcatcaacgctctgtccggcccactgcacggtggcgcaaaccaggctgttctggagatgctcgaagacatcaagaacaaccacggtggcgacgcaaccgcgttcatgaacaaggtcaagaacaaggaagacggcgtccgcctcatgggcttcggacaccgcgtttacaagaactacgatccacgtgcagcaatcgtcaaggagaccgcacacgagatcctcgagcacctcggtggcgacgatcttctggatctggcaatcaagctggaagaaattgcactggctgatgattgcttcatctcccgcaagctctacccgaacgtagacttctacaccggcctgatctaccgcgcaatgggcttcccaactgacttcttcaccgtattgttcgcaatcggtcgtctgccaggatggatcgctcactaccgcgagcagctcggtgcagcagacaacaagatcaaccgcccacgccaggtctacaccggcaaggaatcccgcaagttggttcctcgcgaggagcgctaa

SEQ ID NO: 14 - protein, 437 aa, Artificial Sequence
  ATCC 14067 GltA G413D, K415H AA
MFERDIVATDNNKAVLHYPGGEFEMDIIEASEGNNGVVLGKMLSETGLITFDPGYVSTGSTESKITYIDGDAGILRYRGYDIADLAENATFNEVSYLLINGELPTPDELHKFNDEIRHHTLLDEDFKSQFNVFPRDAHPMATLASSVNILSTYYQDQLNPLDEAQLDKATVRLMAKVPMLAAYAHRARKGAPYMYPDNSLNARENFLRMMFGYPTEPYEIDPIMVKALDKLLILHADHEQNCSTSTVRMIGSAQANMFVSIAGGINALSGPLHGGANQAVLEMLEDIKNNHGGDATAFMNKVKNKEDGVRLMGFGHRVYKNYDPRAAIVKETAHEILEHLGGDDLLDLAIKLEEIALADDYFISRKLYPNVDFYTGLIYRAMGFPTDFFTVLFAIGRLPGWIAHYREQLGAADNHINRPRQVYTGNESRKLVPREER

SEQ ID NO: 15 - DNA, 1314 bp, Artificial Sequence
  ATCC 14067 GltA G413D, K415H NT
atgtttgaaagggatatcgtggctactgataacaacaaggctgtcctgcactaccccggtggcgagttcgaaatggacatcatcgaggcttctgagggtaacaacggtgttgtcctgggcaagatgctgtctgagactggactgatcacttttgacccaggttatgtgagcactggctccaccgagtcgaagatcacctacatcgatggcgatgcgggaatcctgcgttaccgcggctatgacatcgctgatctggctgagaatgccaccttcaacgaggtttcttacctacttatcaacggtgagctaccaaccccagatgagcttcacaagtttaacgacgagattcgccaccacacccttctggacgaggacttcaagtcccagttcaacgtgttcccacgcgacgctcacccaatggcaaccttggcttcctcggttaacattttgtctacctactaccaggatcagctgaacccactcgatgaggcacagcttgataaggcaaccgttcgcctcatggcaaaggttccaatgctggctgcgtacgcacaccgcgcacgcaagggtgctccttacatgtacccagacaactccctcaacgcgcgtgagaacttcctgcgcatgatgttcggttacccaactgagccatacgagatcgacccaatcatggtcaaggctctggacaagctgctcatcctgcacgctgaccacgagcagaactgctccacctccaccgttcgtatgatcggttccgcacaggccaacatgtttgtctccatcgctggtggcatcaacgctctgtccggcccactgcacggtggcgcaaaccaggctgttctggagatgctcgaagacatcaagaacaaccacggtggcgacgcaaccgcgttcatgaacaaggtcaagaacaaggaagacggcgtccgcctcatgggcttcggacaccgcgtttacaagaattacgatccacgtgcagcaatcgtcaaggagaccgcacacgagatcctcgagcacctcggtggcgacgatcttctggatctggcaatcaagctggaagaaattgcactggctgatgattacttcatctcccgcaagctctacccgaacgtagacttctacaccggcctgatctaccgcgcaatgggcttcccaactgacttcttcaccgtattgttcgcaatcggtcgtctgccaggatggatcgctcactaccgcgagcagctcggtgcagcagacaaccacatcaaccgcccacgccaggtctacaccggcaacgaatcccgcaagttggttcctcgcgaggagcgctaa

SEQ ID NO: 16 - protein, 437 aa, Artificial Sequence
  ATCC13032 GltA G413D, K415H AA
MFERDIVATDNNKAVLHYPGGEFEMDIIEASEGNNGVVLGKMLSETGLITFDPGYVSTGSTESKITYIDGDAGILRYRGYDIADLAENATFNEVSYLLINGELPTPDELHKFNDEIRHHTLLDEDFKSQFNVFPRDAHPMATLASSVNILSTYYQDQLNPLDEAQLDKATVRLMAKVPMLAAYAHRARKGAPYMYPDNSLNARENFLRMMFGYPTEPYEIDPIMVKALDKLLILHADHEQNCSTSTVRMIGSAQANMFVSIAGGINALSGPLHGGANQAVLEMLEDIKSNHGGDATEFMNKVKNKEDGVRLMGFGHRVYKNYDPRAAIVKETAHEILEHLGGDDLLDLAIKLEEIALADDYFISRKLYPNVDFYTGLIYRAMGFPTDFFTVLFAIGRLPGWIAHYREQLGAADNHINRPRQVYTGNESRKLVPREER

SEQ ID NO: 17 - DNA, 1314 bp, Artificial Sequence
  ATCC13032 GltA G413D, K415H NT
atgtttgaaagggatatcgtggctactgataacaacaaggctgtcctgcactaccccggtggcgagttcgaaatggacatcatcgaggcttctgagggtaacaacggtgttgtcctgggcaagatgctgtctgagactggactgatcacttttgacccaggttatgtgagcactggctccaccgagtcgaagatcacctacatcgatggcgatgcgggaatcctgcgttaccgcggctatgacatcgctgatctggctgagaatgccaccttcaacgaggtttcttacctacttatcaacggtgagctaccaaccccagatgagcttcacaagtttaacgacgagattcgccaccacacccttctggacgaggacttcaagtcccagttcaacgtgttcccacgcgacgctcacccaatggcaaccttggcttcctcggttaacattttgtctacctactaccaggaccagctgaacccactcgatgaggcacagcttgataaggcaaccgttcgcctcatggcaaaggttccaatgctggctgcgtacgcacaccgcgcacgcaagggtgctccttacatgtacccagacaactccctcaatgcgcgtgagaacttcctgcgcatgatgttcggttacccaaccgagccatacgagatcgacccaatcatggtcaaggctctggacaagctgctcatcctgcacgctgaccacgagcagaactgctccacctccaccgttcgtatgatcggttccgcacaggccaacatgtttgtctccatcgctggtggcatcaacgctctgtccggcccactgcacggtggcgcaaaccaggctgttctggagatgctcgaagacatcaagagcaaccacggtggcgacgcaaccgagttcatgaacaaggtcaagaacaaggaagacggcgtccgcctcatgggcttcggacaccgcgtttacaagaactacgatccacgtgcagcaatcgtcaaggagaccgcacacgagatcctcgagcacctcggtggcgacgatcttctggatctggcaatcaagctggaagaaattgcactggctgatgattacttcatctcccgcaagctctacccgaacgtagacttctacaccggcctgatctaccgcgcaatgggcttcccaactgacttcttcaccgtattgttcgcaatcggtcgtctgccaggatggatcgctcactaccgcgagcagctcggtgcagcagacaaccacatcaaccgcccacgccaggtctacaccggcaacgaatcccgcaagttggttcctcgcgaggagcgctaa

SEQ ID NO: 18 - protein, 437 aa, Artificial Sequence
  ATCC13869 GltA G413D, K415H AA
MFERDIVATDNNKAVLHYPGGEFEMDIIEASEGNNGVVLGKMLSETGLITFDPGYVSTGSTESKITYIDGDAGILRYRGYDIADLAENATFNEVSYLLINGELPTPDELHKFNDEIRHHTLLDEDFKSQFNVFPRDAHPMATLASSVNILSTYYQDQLNPLDEAQLDKATVRLMAKVPMLAAYAHRARKGAPYMYPDNSLNARENFLRMMFGYPTEPYEIDPIMVKALDKLLILHADHEQNCSTSTVRMIGSAQANMFVSIAGGINALSGPLHGGANQAVLEMLEDIKNNHGGDATAFMNKVKNKEDGVRLMGFGHRVYKNYDPRAAIVKETAHEILEHLGGDDLLDLAIKLEEIALADDCFISRKLYPNVDFYTGLIYRAMGFPTDFFTVLFAIGRLPGWIAHYREQLGAADNHINRPRQVYTGKESRKLVPREER

SEQ ID NO: 19 - DNA, 1314 bp, Artificial Sequence
  ATCC13869 GltA G413D, K415H NT
atgtttgaaagggatatcgtggctactgataacaacaaggctgtcctgcactaccccggtggcgagttcgaaatggacatcatcgaggcttctgagggtaacaacggtgttgtcctgggcaagatgctgtctgagactggactgatcacttttgacccaggttatgtgagcactggctccaccgagtcgaagatcacctacatcgatggcgatgcgggaatcctgcgttaccgcggctatgacatcgctgatctggctgagaatgccaccttcaacgaggtttcttacctacttatcaacggtgagctaccaaccccagatgagcttcacaagtttaacgacgagattcgccaccacacccttctggacgaggacttcaagtcccagttcaacgtgttcccacgcgacgctcacccaatggcaaccttggcttcctcggttaacattttgtctacctactaccaggatcagctgaacccactcgatgaggcacagcttgataaggcaaccgttcgcctcatggcaaaggttccaatgctggctgcgtacgcacaccgcgcacgcaagggtgctccttacatgtacccagacaactccctcaacgcgcgtgagaacttcctgcgcatgatgttcggttacccaaccgagccatacgagatcgacccaatcatggtcaaggctctggacaagctgctcatcctgcacgctgaccacgagcagaactgctccacctccaccgttcgtatgatcggttccgcacaggccaacatgtttgtctccatcgctggtggcatcaacgctctgtccggcccactgcacggtggcgcaaaccaggctgttctggagatgctcgaagacatcaagaacaaccacggtggcgacgcaaccgcgttcatgaacaaggtcaagaacaaggaagacggcgtccgcctcatgggcttcggacaccgcgtttacaagaactacgatccacgtgcagcaatcgtcaaggagaccgcacacgagatcctcgagcacctcggtggcgacgatcttctggatctggcaatcaagctggaagaaattgcactggctgatgattgcttcatctcccgcaagctctacccgaacgtagacttctacaccggcctgatctaccgcgcaatgggcttcccaactgacttcttcaccgtattgttcgcaatcggtcgtctgccaggatggatcgctcactaccgcgagcagctcggtgcagcagacaaccacatcaaccgcccacgccaggtctacaccggcaaggaatcccgcaagttggttcctcgcgaggagcgctaa

SEQ ID NO: 20 - protein, 172 aa, Unknown
  IlvN AA
MANSDVTRHILSVLVQDVDGIISRVSGMFTRRAFNLVSLVSAKTETLGINRITVVVDADELNIEQITKQLNKLIPVLKVVRLDEETTIARAIMLVKVSADSTNRPQIVDAANIFRARVVDVAPDSVVIESTGTPGKLRALLDVMEPFGIRELIQSGQIALNRGPKTMAPAKI

SEQ ID NO: 21 - DNA, 520 bp, Unknown
  IlvN NT
atggctaattctgacgtcacccgccacatcctgtccgtactcgttcaggacgtagacggaatcatttcccgcgtatcaggtatgttcacccgacgcgcattcaacctcgtgtccctcgtgtctgcaaagaccgaaacactcggcatcaaccgcatcacggttgttgtcgacgccgacgagctcaacattgagcagatcaccaagcagctcaacaagctgatccccgtgctcaaagtcgtgcgacttgatgaagagaccaccatcgcccgcgcaatcatgctggttaaggtctctgcggatagcaccaaccgtccgcagatcgtcgacgccgcgaacatcttccgcgcccgagtcgtcgacgtggctccagactctgtggttattgaatccacaggcaccccaggcaagctccgcgcactgcttgatgtgatggaaccattcggaatccgcgaactgatccaatccggacagattgcactcaaccgcggtccgaagaccatggctccggccaagatctaaa

SEQ ID NO: 22 - protein, 172 aa, Artificial Sequence
  IlvN A42V AA
MANSDVTRHILSVLVQDVDGIISRVSGMFTRRAFNLVSLVSVKTETLGINRITVVVDADELNIEQITKQLNKLIPVLKVVRLDEETTIARAIMLVKVSADSTNRPQIVDAANIFRARVVDVAPDSVVIESTGTPGKLRALLDVMEPFGIRELIQSGQIALNRGPKTMAPAKI

SEQ ID NO: 23 - DNA, 519 bp, Artificial Sequence
  IlvN A42V NT
atggctaattctgacgtcacccgccacatcctgtccgtactcgttcaggacgtagacggaatcatttcccgcgtatcaggtatgttcacccgacgcgcattcaacctcgtgtccctcgtgtctgtaaagaccgaaacactcggcatcaaccgcatcacggttgttgtcgacgccgacgagctcaacattgagcagatcaccaagcagctcaacaagctgatccccgtgctcaaagtcgtgcgacttgatgaagagaccaccatcgcccgcgcaatcatgctggttaaggtctctgcggatagcaccaaccgtccgcagatcgtcgacgccgcgaacatcttccgcgcccgagtcgtcgacgtggctccagactctgtggttattgaatccacaggcaccccaggcaagctccgcgcactgcttgatgtgatggaaccattcggaatccgcgaactgatccaatccggacagattgcactcaaccgcggtccgaagaccatggctccggccaagatctaa

SEQ ID NO: 24 - protein, 127 aa, Artificial Sequence
  General formula 1
  MISC_FEATURE (1): Xaa is N or S.
  MISC_FEATURE (9): Xaa is A or E.
  MISC_FEATURE (73): Xaa is Y or C.
  MISC_FEATURE (127): Xaa is K or H.
XNHGGDATXFMNKVKNKEDGVRLMGFGHRVYKNYDPRAAIVKETAHEILEHLGGDDLLDLAIKLEEIALADDXFISRKLYPNVDFYTGLIYRAMGFPTDFFTVLFAIGRLPGWIAHYREQLGAADNX

SEQ ID NO: 25 - DNA, 44 bp, Artificial Sequence
  primer 1
tcgagctcggtacccccgttcgtatgatcggttccgcacaggcc

SEQ ID NO: 26 - DNA, 31 bp, Artificial Sequence
  primer 2
cgtgggcggttgatcttgttgtctgctgcac

SEQ ID NO: 27 - DNA, 31 bp, Artificial Sequence
  primer 3
gtgcagcagacaacaagatcaaccgcccacg

SEQ ID NO: 28 - DNA, 46 bp, Artificial Sequence
  primer 4
ctctagaggatccccgccgtaagcagcctctggtggaatggtcagc

SEQ ID NO: 29 - DNA, 24 bp, Artificial Sequence
  primer 5
atgtttgaaagggatatcgtggct

SEQ ID NO: 30 - DNA, 22 bp, Artificial Sequence
  primer 6
ttagcgctcctcgcgaggaacc

SEQ ID NO: 31 - DNA, 33 bp, Artificial Sequence
  primer 7
tcgagctcggtacccccgcgtcaccaaagcgga

SEQ ID NO: 32 - DNA, 30 bp, Artificial Sequence
  primer 8
gtccctcgtgtctgtaaagaccgaaacact

SEQ ID NO: 33 - DNA, 30 bp, Artificial Sequence
  primer 9
agtgtttcggtctttacagacacgagggac

SEQ ID NO: 34 - DNA, 35 bp, Artificial Sequence
  primer 10
ctctagaggatccccttagatcttggccggagcca

SEQ ID NO: 35 - DNA, 18 bp, Artificial Sequence
  primer 11
ccgcgtcaccaaagcgga

SEQ ID NO: 36 - DNA, 20 bp, Artificial Sequence
  primer 12
ttagatcttggccggagcca

SEQ ID NO: 37 - DNA, 31 bp, Artificial Sequence
  primer 13
cgtgggcggttgatgtggttgtctgctgcac

SEQ ID NO: 38 - DNA, 31 bp, Artificial Sequence
  primer 14
gtgcagcagacaaccacatcaaccgcccacg